European Patent Application EP 4 349 995 A1, published April 10, 2024. Title: METHOD FOR USING REDUCTION TO PREPARE (S)-NICOTINE. Applicant: PORTON PHARMA SOLUTIONS LTD. The sequence listing filed with the application follows.

SEQUENCE LISTING (22 sequences)

SEQ ID NO: 1 - protein, 260 aa, Artificial Sequence
  Fully synthetic
MYKDLEGKVVVITGSSTGLGKSMAIRFATEKAKVVVNYRSKEDEANSVLEEIKKVGGEAIAVKGDVTVESDVINLVQSAIKEFGKLDVMINNAGLENPVSSHEMSLSDWNKVIDTNLTGAFLGSREAIKYFVENDIKGTVINMSSVHEKIPWPLFVHYAASKGGMKLMTETLALEYAPKGIRVNNIGPGAINTPINAEKFADPEQRADVESMIPMGYIGEPEEIAAVAAWLASSEASYVTGITLFADGGMTQYPSFQAGR

SEQ ID NO: 2 - protein, 292 aa, Artificial Sequence
  Fully synthetic
MRHLSVIGLGAMGSALATTLLKAGHPVTVWNRSAAKAAPLQALGATLAPSVGEAIAASDITLVCVDNYAVSQQLLDEASDAVAGKLLVQLSTGSPQGARSLESWCHTRGARYLDGAILCFPDQIGTTDASIICSGASTAFSEAEPVLRLLAPPLDHVAEAVGAAAAQDCAVAAYFAGGLLGALHGALICEVEGLPVAKVCAQFSELSPILGGDVAHLGKTLASGDFDHPYASLKTWSAAISRLAGHATDAGIDSRFPRFAADLFEEGVAQGFGQQEVSALIKVLRARNGAAQ

SEQ ID NO: 3 - protein, 292 aa, Artificial Sequence
  Fully synthetic
MRHLSVIGLGAMGSALATTLLKAGHPVTVWNRSAAKAAPLQALGATLAPSVGAAIAASDITLVCVDNYAVSQLLLDEASDAVAGKLLVQLSTGSPQGARALESWSHARGARYLDGAILCFPAQIGTSDASIICSGASAAFSEAEPVLSLLAPTLDHVAEAVGAAAAQDCAVAAYFAGGLLGALHGALICEAEGLPVAKVCAQFSELSPILGGDVAHLGKTLASGDFDHPYASLKTWSAAISRLAGHATDAGIDSRFPRFAADLFEEGVAQGFGQQEVSALIKVLRARNGAAQ

SEQ ID NO: 4 - protein, 258 aa, Artificial Sequence
  Fully synthetic
MRHLSVIGLGAMGSALATTLIKGGHPVTVWNRSAAKAAPLQALGATLAPSVGAAIAASDITLVCVDNYAVSQQLLDEARDAVAGKLLVQLSTGSPQGARALESWSHARGARYLDGAILCFPDQIGTSDASIICSGASAAYFAGGLLGALHGALICEAEGLPVAKVCAQFSELSPILGGDVAHLGKTLASGDFDHPYASLKTWSAAISRLAGHATDAGIDSRFPRFAADLFEEGVAQGFGQQEVSALIKVLRARNGAAL

SEQ ID NO: 5 - protein, 292 aa, Artificial Sequence
  Fully synthetic
MRPISVIGLGAMGSALATTLLKAGHPVTVWNRSAAKATPLIALGAILAPSVSEAIAAGDITLICVDNYAVSQQLLDEASNAVTGKLVVQLSTGSPLGARTLESWCHARGACYLDGAILCFPDQIGTTDASIICSGANAAFREAEPVLRLLAPTLEHVAEAVGAAAAQDCAVAAYFAGGLLGALHGALICEAEGLPVAKVCAQFSELSPILGGDVAHLGKTLASGDFDHPYASLKTWSAAISRLTDHAADAGIDNSFPRFAADLFEEGVEQGLGQQEVSALIKVLRARNGAAQ

SEQ ID NO: 6 - protein, 292 aa, Artificial Sequence
  Fully synthetic
MRHLSVIGLGAMGSALATTLIKAGHPVTVWNRSAAKSAPLQALGATLAPSVGAAIAASDITLVCVDNYAVSQQLLDEASDAVAGKQLVQLSTGSPQGARALESWSHARGARYLDGAILCFPDQIGTSDASIICSGANTAFSDAEPVLRLLAPTLDHVAEAVGAAAAQDCAVAAYFAGGLLGALHGALICEAEGLPVTKVCAQFSELSPILGGDVAHLGKTLASGDFDHPYASLKTWSAAISRLAGHATDAGIDSRFPRFAADLFEEGVAQGFGQQEVSALIKVLRARNGAAQ

SEQ ID NO: 7 - protein, 276 aa, Artificial Sequence
  Fully synthetic
MGTALVEAFLAGGHATTVWNRTPGKADGVVARGAVVAETVAEAVAASPLVVVCLWDDAVVRDVLHPVADALAGRVVVNLTNGTPAQAREMAAWAAEHGVEYVDGGIMAIPPGIGTEHAFVLYSGAEAAFEAHREVLERLGAAKYLGADAGLAALFDLALLSGMYGTFAGLWHSLAMVRTENVSAAEFVPMLGPWMQAMIGGNLDRLAHQLDTGDYGHEVVSNLAMQAAAFPNIVQASLDQGIRPDLMAPIQRLMDQAVAAGHGAEDVAVVVDLLKN

SEQ ID NO: 8 - protein, 291 aa, Artificial Sequence
  Fully synthetic
MKPTLTVIGAGRMGSALIKAFLQSGYTTTVWNRTKAKSEPLAKLGAHLADTVRDAVKRSDIIVVNVLDYDTSDQLLRQDEVTRELRGKLLVQLTSGSPALAREQETWARQHGIDYLDGAIMATPDFIGQAECALLYSGSAALFEKHRAVLNVLGGATSHVGEDVGHASALDSALLFQMWGTLFGTLQALAISRAEGIPLEKTTAFIKLTEPVTQGAVADVLTRVQQNRLTADAQTLASLEAHNVAFQHLLALCEERNIHRGVADAMYSVIREAVKAGHGKDDFAILTRFLK

SEQ ID NO: 9 - protein, 329 aa, Artificial Sequence
  Fully synthetic
MVSSPYLNVTAYPKVRNLPWPVPGPIRVASQILELRPMTTIGFLGAGRMGSALVKSLLEAGHSVHVWNRTAEKAQALADFGAVPEPSAERAAGPAEIVIVNLLDYEASDAELRKPDVAEALKGKLLVQLTSGSPKTARETGRWAGDHGIAYLDGAIMATPNFIGGAETVILYSGSKTHFEKHEGLFKALGGKSAFVGEDFGTASALDSALLSQMWGTLFGTLQALAVCRAEGIEHDVYAGFLMSAQPMIDGAQQDLMERIRDGRDLADAQTLATVAVHNVAFHHLRDLIADRDLNPAFGDALGSLLETALRNDHQDDDFAVLARFMGAK

SEQ ID NO: 10 - protein, 293 aa, Artificial Sequence
  Fully synthetic
MTDLGKSAVTVLGLGAMGTALAEALLAAGHPTTVWNRSPARTAGPAQRGAAVAAATAEAIAASRLIVVCLLDHTSVHAVLDGQELTGRIVVNLTSGTPGQARELDARVAERGGDHLDGAVLAVPSMIGTPDASVLYSGSRGAFDTHRPVLEVFGAADYVGADPGAASLQDAALLSAMYGQVAGVLHAFALVRSAGVTATEFLPRLVGWLTAMGGFPADAARRIDARAYADDVDAALTMQVTAVRNLVRAAREQGVSAELIAPLVPVMQRRIDDGDGGDDLAALVEVITAEEVA

SEQ ID NO: 11 - protein, 290 aa, Artificial Sequence
  Fully synthetic
MTDKPPVTVLGLGAMGTALARTLLNAGYPTTVWNRTASKTAPLTELGAHAADSPADAIARGELVLACLLDYDSVHQTLAGTGDALRGKAFVNLTNGTPEQARALAGKLDTAYLDGGIMAVPPMIGSPGAFLFYSGEIAVFEQYRPVLESFGEAIEVGTDPGLAALHDLALLSAMYGMFGGVLQAFALTGSAGVSAASLAPLLHRWLDGMSGFIAQSAAQLDSGDFATGVVSNLAMQDTGFANLFRAAKEQGISTGQLEPLGALIRRRVEDGHGAEDLAGIVEYLKIGANA

SEQ ID NO: 12 - protein, 292 aa, Artificial Sequence; identical to SEQ ID NO: 3
  Fully synthetic

SEQ ID NO: 13 - protein, 292 aa, Artificial Sequence
  Fully synthetic
MRHLSVIGLGAMGSALATTLLKAGHPVTVWNRSAAKAAPLQALGATLAPSVGAAIAASDITLVCVDNYAVSQVLLDEASDAVAGKLLVQLSTGSPQGARALESWSHARGARYLDGAILCFPAQIGTSDASIICSGASAAFSEAEPVLSLLAPTLDHVAEAVGAAAAQDCAAAAYFAGGLLGALHGALICEAEGLPVAKVCAQFSELSPILGGDVAHLGKTLASGDFDHPYASLKTWSAAISRLAGHATDAGIDSRFPRFAADLFEEGVAQGFGQQEVSALIKVLRARNGAAQ

SEQ ID NO: 14 - protein, 292 aa, Artificial Sequence
  Fully synthetic
MRHLSVIGLGAMGSALATTLLKAGHPVTVWNRSAAKAAPLQALGATLAPSVGAAIAASDITLVCVDNYAVSQQLLDEASDAVAGKLLVQLSTGSPQGARALESWSHARGARYLDGAILCFPAQIGTSDASIICSGASAAFSEAEPVLRLLAPTLDHVAEAVGAAAAQDCAVAAYFAGGLLGALHGALICEAEGLPVAKVCAQFSELSPILGGDVAHLGKTLASGDFDHPYASLKTWSAAISRLAGHATDAGIDSRFPRFAADLFEEGVAQGFGQQEVSALIKVLRARNGAAQ

SEQ ID NO: 15 - protein, 292 aa, Artificial Sequence
  Fully synthetic
MRHLSVIGLGAMGSALATTLLKAGHPVTVWNRSAAKAAPLQALGATLAPSVGAAIAASDITLVCVDNYAVSQQLLDEASDAVAGKLLVQLSTGSPQGARALESWSHARGARYLDGAILCFPAQIGTSDASIICSGASAAFSEAEPVLRLLAPTLDHVAEAVGAAAAQDCAVAAYFAGGLLGALHGALICEAEGLPVAKVCAQFSELSPILGGDVAHLGKTLASGDFDHPGASLKTWSAAISRLAGHATDAGIDSRFPRFAADLFEEGVAQGFGQQEVSALIKVLRARNGAAQ

SEQ ID NO: 16 - protein, 292 aa, Artificial Sequence
  Fully synthetic
MRHLSVIGLGAMGSALATTLLKAGHPVTVWNRSAAKAAPLQALGATLAPSVGAAIARSDITLVCVDNYAVSQLLLDEASDAVAGKLLVQLSTGSPQGARALESWSHARGARYLDGAILCFPAQIGTSDASIICSGASAAFSEAEPVLSLLAPTLDHVAEAVGAAAAQDCAAVAYFGGGLLGALHGALICEAEGLPVAKVCAQFSELSPILGGDVAHLGKTLASGDFDHPTASLKTWSAAIGRLAGHATDAGIDSRFPRFAADLFEEGVAQGFGQQEVSALIKVLRARNGAAQ

SEQ ID NO: 17 - protein, 292 aa, Artificial Sequence
  Fully synthetic
MRHLSVIGLGAMGSALATTLLKAGHPVTVWNRSAAKAAPLQALGATLAPSVGAAIARSDITLVCVDNYAVSQLLLDEASDAVAGKLLVQLSTGSPQGARALESWSHARGARYLDGAILCFPAQIGTSDASIICSGASAAFSEAEPVLSLLAPTLDHVAEAVGAAAAQDCAAVAYFGGGLLGALHGALICEAEGLPVAKVCAQFSELSPILGGDVAHLGKTLASGDFDHPYASLKTWSAAIGRLAGHATDAGIDSRFPRFAADLFEEGVAQGFGQQEVSALIKVLRARNGAAQ

SEQ ID NO: 18 - protein, 292 aa, Artificial Sequence
  Fully synthetic
MRHLSVIGLGAMGSALATTLLKAGHPVTVWNRSAAKAAPLQALGATLAPSVGAAIARSDITLVCVDNYAVSQLLLDEASDAVAGKLLVQLSTGSPQGARALESWSHARGARYLDGAILCFPAQIGTSDASIICSGASAAFSEAEPVLSLLAPTLDHVAEAVGAAAAQDCAAAAYFGGGLLGALHGALICEAEGLPVAKVCAQFSELSPILGGDVAHLGKTLASGDFDHPYASLKTWSAAIGRLAGHATDAGIDSRFPRFAADLFEEGVAQGFGQQEVSALIKVLRARNGAAQ

SEQ ID NO: 19 - protein, 292 aa, Artificial Sequence
  Fully synthetic
MRHLSVIGLGAMGSALATTLLKAGHPVTVWNRSAAKAAPLQALGATLAPSVGAAIARSDITLVCVDNYAVSQLLLDEASDAVAGKLLVQLSTGSPQGARALESWSHARGARYLDGAILCFPAQIGTSDASIICSGASAAFSEAEPVLSLLAPTLDHVAEAVGAAAAQDCAVVAYFGGGLLGALHGALICEAEGLPVAKVCAQFSELSPILGGDVAHLGKTLASGDFDHPYASLKTWSAAIGRLAGHATDAGIDSRFPRFAADLFEEGVAQGFGQQEVSALIKVLRARNGAAQ

SEQ ID NO: 20 - protein, 292 aa, Artificial Sequence
  Fully synthetic
MRHLSVIGLGAMGSALATTLLKAGHPVTVWNRSAAKAAPLQALGATLAPSVGAAIARSDITLVCVDNYAVSQQLLDEASDAVAGKLLVQLSTGSPQGARALESWSHARGARYLDGAILCFPAQIGTSDASIICSGASAAFSEAEPVLRLLAPTLDHVAEAVGAAAAQDCAVAAYFGGGLLGALHGALICEAEGLPVAKVCAQFSELSPILGGDVAHLGKTLASGDFDHPYASLKTWSAAISRLAGHATDAGIDSRFPRFAADLFEEGVAQGFGQQEVSALIKVLRARNGAAQ

SEQ ID NO: 21 - protein, 292 aa, Artificial Sequence
  Fully synthetic
MRHLSVIGLGAMGSALATTLLKAGHPVTVWNRSAAKAAPLQALGATLAPSVGAAIARSDITLVCVDNYAVSQQLLDEASDAVAGKLLVQLSTGSPQGARALESWSHARGARYLDGAILCFPAQIGTSDASIICSGASAAFSEAEPVLRLLAPTLDHVAEAVGAAAAQDCAVAAYFGGGLLGALHGALICEAEGLPVAKVCAQFSELSPILGGDVAHLGKTLASGDFDHPYASLKTWSAAIARLAGHATDAGIDSRFPRFAADLFEEGVAQGFGQQEVSALIKVLRARNGAAQ

SEQ ID NO: 22 - protein, 292 aa, Artificial Sequence
  Fully synthetic
MRHLSVIGLGAMGSALATTLLKAGHPVTVWNRSAAKAAPLQALGATLAPSVGAAIARSDITLVCVDNYAVSQQLLDEASDAVAGKLLVQLSTGSPQGARALESWSHARGARYLDGAILCFPAQIGTSDASIICSGASAAFSEAEPVLRLLAPTLDHVAEAVGAAAAQDCAVAAYFGGGLLGALHGALICEAEGLPVAKVCAQFSELSPILGGDVAHLGKTLASGDFDHPTASLKTWSAAISRLAGHATDAGIDSRFPRFAADLFEEGVAQGFGQQEVSALIKVLRARNGAAQ